European Patent Application EP 4 144 362 A1, published March 8, 2023. Title: COMPOSITIONS COMPRISING SHORT-ACTING HORMONES FOR TREATING OR PREVENTING OBESITY AND PUMPS COMPRISING SAID COMPOSITION. Applicant: ADOCIA. Application EP21195161.1. The sequence listing filed with the application follows.

SEQUENCE LISTING (54 sequences)

SEQ ID NO: 1 - protein, 37 aa, Homo sapiens [sequence omitted]

SEQ ID NO: 2 - protein, 37 aa, Artificial Sequence
  Pramlintide
KCNTATCATQRLANFLVHSSNNFGPILPPTNVGSNTY

SEQ ID NO: 3 - protein, 37 aa, Artificial Sequence
  Formula A1
  VARIANT 1: Xaa1 is absent or independently selected from Ala, Cys, Glu, Gly, His, Arg, Ser and Lys
  VARIANT 3: Xaa3 is independently selected from Gly, His, Arg, Ser and Asn
  VARIANT 14: Xaa14 is independently selected from Asp, Glu, His, Asn, Arg, Gly, Ala, Ser, Lys, Thr and Cys
  VARIANT 17: Xaa17 is independently selected from His, Arg, Lys and Val
  VARIANT 18: Xaa18 is independently selected from Arg, Lys and His
  VARIANT 21: Xaa21 is independently selected from Ala, Lys, Gln, Ser, Asn and Pro
  VARIANT 22: Xaa22 is independently selected from Glu, Gln, Ser, Thr and Asn
  VARIANT 25: Xaa25 is independently selected from Pro and Ala
  VARIANT 26: Xaa26 is independently selected from Pro, Arg and Ile
  VARIANT 27: Xaa27 is independently selected from Pro and Leu
  VARIANT 28: Xaa28 is independently selected from Pro and Ser
  VARIANT 29: Xaa29 is independently selected from Pro and Ser
  VARIANT 31: Xaa31 is independently selected from Ser, Glu, Asp, Pro and Asn
  VARIANT 34: Xaa34 is independently selected from Pro, His, Lys, Arg and Ser
  VARIANT 35: Xaa35 is independently selected from His, Arg, Lys, Asp, Glu, Gln and Asn
  VARIANT 37: Xaa37 is independently selected from Pro and Tyr
XCXTATCATQRLAXFLXXSSXXFGXXXXXTXVGXXTX

SEQ ID NO: 4 - protein, 37 aa, Artificial Sequence
  Formula B1
  VARIANT 1: Xaa(-1) is absent or Glu
  VARIANT 2: Xaa1 is absent or selected from the group consisting of Glu or Ala
  VARIANT 3: Xaa2 is selected from the group consisting of Leu, Ala or Pro
  VARIANT 4: Xaa3 is selected from the group consisting of Ser or Pro
  VARIANT 5: Xaa4 is selected from the group consisting of Glu, Pro, Lys, Gln or Gly
  VARIANT 6: Xaa5 is selected from the group consisting of Leu, Val, or Ile
  VARIANT 7: Xaa6 is Ser, Thr or His
  VARIANT 8: Xaa7 is Thr
  VARIANT 9: Xaa8 is selected from the group consisting of Leu or Ala
  VARIANT 10: Xaa9 is selected from the group consisting of Ala, Val, Ile, Ser or Thr
  VARIANT 11: Xaa10 is selected from the group consisting of Leu, Ala, Ile, His or Val
  VARIANT 12: Xaa11 is Gly
  VARIANT 13: Xaa12 is selected from the group consisting of Arg, His or Lys
  VARIANT 14: Xaa13 is Leu
  VARIANT 15: Xaa14 is selected from the group consisting of Ser, Thr or Glu
  VARIANT 16: Xaa15 is selected from the group consisting of Ala, Gln, Glu, D-Glu or Thr
  VARIANT 17: Xaa16 is selected from the group consisting of Arg, Glu, Lys or Gln
  VARIANT 18: Xaa17 is selected from the group consisting of Leu or Ile
  VARIANT 19: Xaa18 is selected from the group consisting of His or Ala
  VARIANT 20: Xaa19 is selected from the group consisting of Glu, Arg or Lys
  VARIANT 21: Xaa20 is selected from the group consisting of Leu, Ile or Val
  VARIANT 22: Xaa21 is selected from the group consisting of Ala, Gln, Ser, Glu or Thr
  VARIANT 23: Xaa22 is Thr
  VARIANT 24: Xaa23 is selected from the group consisting of Thr, Tyr or Leu
  VARIANT 25: Xaa24 is Pro
  VARIANT 26: Xaa25 is selected from the group consisting of Arg, Pro, His or Lys
  VARIANT 27: Xaa26 is Thr
  VARIANT 28: Xaa27 is selected from the group consisting of Glu, Gln, Gly or Lys
  VARIANT 29: Xaa28 is selected from the group consisting of Thr or Pro
  VARIANT 30: Xaa29 is Gly
  VARIANT 31: Xaa30 is selected from the group consisting of Pro, Ser or Thr
  VARIANT 32: Xaa31 is selected from the group consisting of Glu, Gln, Gly, Ala, Pro or Lys
  VARIANT 33: Xaa32 is selected from the group consisting of Thr, Ser, His, Pro or Ala
  VARIANT 34: Xaa33 is selected from the group consisting of Pro, Tyr, His, Phe, Leu, Ser, Gly or Ala
  VARIANT 35: Xaa34 is absent or Gly
  VARIANT 36: Xaa35 is absent or Thr
  VARIANT 37: Xaa36 is absent or Tyr
XXXXXXXXXXXXXXXXXXXXXXXXXXXXXXXXXXXXX

SEQ ID NO: 5 - protein, 38 aa, Artificial Sequence
  Formula C1
  VARIANT 1: Xaa0 is a basic amino acid or is absent
  VARIANT 2: Xaa1 is a basic amino acid or is selected from the group consisting of Ala and Trp
  DISULFID 3..8
  VARIANT 4: Xaa3 is selected from the group consisting of Asn, Gly, Ser, Pro, Asp and Glu
  VARIANT 11: Xaa10 is selected from the group consisting of Gln, Gly, Ala, Ser, Leu, Thr, Pro, Asp and Glu
  VARIANT 13: Xaa12 is selected from the group consisting of Leu and DLeu
  VARIANT 15: Xaa14 is selected from the group consisting of Glu, DGlu, Asp and DAsp
  VARIANT 17: Xaa16 is selected from the group consisting of Leu and DLeu, or is absent
  VARIANT 18: Xaa17 is selected from the group consisting of His, DHis, Val, DVal, Arg, DArg, Lys, DLys, Orn, DOrn, Dap and Dab, or is absent
  VARIANT 19: Xaa18 is selected from the group consisting of His, DHis, Arg, DArg, Dap and Dab, or is absent
  VARIANT 20: Xaa19 is selected from the group consisting of Ser and DSer, or is absent
  VARIANT 21: Xaa20 is selected from the group consisting of Ser and DSer, or is absent
  VARIANT 22: Xaa21 is selected from the group consisting of Asn, DAsn, Glu, DGlu, Asp, DAsp, Ser and DSer, or is absent
  VARIANT 23: Xaa22 is selected from the group consisting of Asn, DAsn, Glu, DGlu, Asp, DAsp, Ser and DSer, or is absent
  VARIANT 24: Xaa23 is selected from the group consisting of Phe and DPhe, or is absent
  VARIANT 25: Xaa24 is selected from the group consisting of Gly(Me), Ala(Me), DAla(Me), Ile(Me), DIle(Me), Ala, DAla, Pro and DPro,or is absent
  VARIANT 26: Xaa25 is selected from the group consisting of Ala, DAla, Pro and DPro, or is absent;
  VARIANT 27: Xaa26 is selected from the group consisting of Gly(Me), Ile(Me), DIle(Me), Ile and DIle, or is absent
  VARIANT 28: Xaa27 is selected from the group consisting of Leu and DLeu, or is absent
  VARIANT 29: Xaa28 is selected from the group consisting of Ser, DSer, Pro, DPro, Ser(Me) and DSer(Me), or is absent
  VARIANT 30: Xaa29 is selected from the group consisting of Ser, DSer, Pro, DPro, Ser(Me) and DSer(Me), or is absent
  VARIANT 31: Xaa30 is selected from the group consisting of Thr and DThr, or is absent
  VARIANT 32: Xaa31 is selected from the group consisting of Asn, DAsn, Glu, DGlu, Asp and DAsp, or is absent
  VARIANT 36: Xaa35 is selected from the group consisting of His, DHis, Asn, DAsn, Glu, DGlu, Asp and DAsp, or is absent
  VARIANT 38: Xaa37 is selected from the group consisting of Tyr, DTyr, Pro, DPro, Hyp, Phe, Ser, Gly, Ala, Val, Ile, Leu, Thr, Tyr(Me), Gly(Me), Ala(Me), Ile(Me), Aze, Pip, Apr, Php and Bep, or is absent
XXCXTATCATXRXAXFXXXXXXXXXXXXXXXXVGSXTX

SEQ ID NO: 6 - protein, 37 aa, Artificial Sequence
  Formula D1
  VARIANT 3: Xaa3 is selected from the group consisting of Asn, Gly, Pro and Gln
  VARIANT 10: Xaa10 is selected from the group consisting of Gln, Asp and Glu
  VARIANT 14: Xaa14 is selected from the group consisting of Asp, His, Asn and Aad
  VARIANT 17: Xaa17 is selected from the group consisting of His, Asn, Gln, Glu, Thr, Val, Lys and Aad
  VARIANT 19..20: Xaa19-Xaa20 is selected from the group consisting of Ser-Ser, Val-Val, Ser-Val and Val-Ser, or is absent
  SITE 21..22: Xaa21-Xaa22 are absent
  MOD_RES 24: METHYLATION MeGly
  MOD_RES 26: METHYLATION MeIle
  VARIANT 31: Xaa31 is selected from the group consisting of Asp, Glu and Asn
  VARIANT 35: Xaa35 is selected from the group consisting of Asp, Glu, Asn, Ser, Phe, Orn, Aad, Gly and Thr
  VARIANT 37: Xaa37 is selected from the group consisting of Pro, Apr and Hyp
RCXTATCATXRLAXFLXRXXXXFGAILSSTXVGSXTX

SEQ ID NO: 7 - protein, 37 aa, Artificial Sequence
  Formula E1
  VARIANT 1: Xaa1 is selected from the group consisting of Arg, Lys and Glu
  STRAND 2..7: Xaa2 and Xaa7 are amino acid residues whose side chains together form a lactam bridge;
  VARIANT 3: Xaa3 is selected from the group consisting of Gly, Gln and Pro
  VARIANT 4: Xaa4 is selected from the group consisting of Thr and Glu
  VARIANT 5: Xaa5 is selected from the group consisting of Ala and Leu
  VARIANT 6: Xaa6 is selected from the group consisting of Thr and Ser;
  VARIANT 10: Xaa10 is selected from the group consisting of Glu and Gln
  VARIANT 14: Xaa14 is selected from the group consisting of Aad, His, Asp, Asn and Arg
  VARIANT 17: Xaa17 is selected from the group consisting of Gln, His and Thr
  VARIANT 19..20: Xaa19-Xaa20 is selected from Ser-Ser, Thr-Thr, Ala-Thr, Ala-Ala, Gly-Thr, Gly-Gly and Ala-Asn or is absent
  SITE 21..22: Xaa21-Xaa22 are absent
  MOD_RES 24: METHYLATION MeGly
  MOD_RES 26: METHYLATION MeIle
  VARIANT 27: Xaa27 is selected from the group consisting of Leu and Pro
  VARIANT 32: Xaa32 is selected from the group consisting of Val and Thr
  VARIANT 35: Xaa35 is selected from the group consisting of Asn and Ser
  VARIANT 37: Xaa37 is selected from the group consisting of Hyp and Pro
XXXXXXXATXRLAXFLXRXXXXFGAIXSSTEXGSXTX

SEQ ID NO: 8 - protein, 37 aa, Artificial Sequence
  Formula A1-1
  VARIANT 1: Xaa1 is absent or independently selected from Ala, Cys, Glu, Gly, His, Arg, Ser and Lys
  VARIANT 3: Xaa3 is independently selected from Gly, His, Arg, Ser and Asn
  VARIANT 14: Xaa14 is Glu
  VARIANT 17: Xaa17 is independently selected from His, Arg, Lys and Val
  VARIANT 18: Xaa18 is independently selected from Arg, Lys and His
  VARIANT 21: Xaa21 is independently selected from Ala, Lys, Gln, Ser and Asn
  VARIANT 22: Xaa22 is independently selected from Glu, Gln, Ser, Thr and Asn
  VARIANT 26: Xaa26 is independently selected from Pro, Arg and Ile
  VARIANT 31: Xaa31 is independently selected from Ser, Glu, Asp and Asn;
  VARIANT 35: Xaa35 is independently selected from His, Arg, Lys, Asp and Glu
  VARIANT 37: Xaa37 is independently selected from Pro and Tyr
XCXTATCATQRLAXFLXXSSXXFGPXLPPTXVGSXTX

SEQ ID NO: 9 - protein, 37 aa, Artificial Sequence; identical to SEQ ID NO: 8
  Formula A1-2
  VARIANT 1: Xaa1 is absent or independently selected from Ala, Cys, Glu, Gly, His, Arg, Ser and Lys
  VARIANT 3: Xaa3 is independently selected from Gly, His, Arg, Ser and Asn
  VARIANT 14: Xaa14 is independently selected from Glu and Asn
  VARIANT 17: Xaa17 is Arg
  VARIANT 18: Xaa18 is independently selected from Arg, Lys and His
  VARIANT 21: Xaa21 is independently selected from Ala, Lys, Gln, Ser and Asn
  VARIANT 22: Xaa22 is independently selected from Glu, Gln, Ser, Thr and Asn
  VARIANT 26: Xaa26 is independently selected from Pro, Arg and Ile
  VARIANT 31: Xaa31 is independently selected from Ser, Glu, Asp and Asn
  VARIANT 35: Xaa35 is independently selected from His, Arg, Lys, Asp and Glu
  VARIANT 37: Xaa37 is independently selected from Pro and Tyr

SEQ ID NO: 10 - protein, 37 aa, Artificial Sequence; identical to SEQ ID NO: 8
  Formula A1-3
  VARIANT 1: Xaa1 is absent or independently selected from Ala, Cys, Glu, Gly, His, Arg, Ser and Lys
  VARIANT 3: Xaa3 is independently selected from Gly, His, Arg, Ser and Asn
  VARIANT 14: Xaa14 is independently selected from Glu and Asn
  VARIANT 17: Xaa17 is independently selected from His, Arg, Lys and Val
  VARIANT 18: Xaa18 is independently selected from Arg, Lys and His
  VARIANT 21: Xaa21 is independently selected from Ala, Lys, Gln, Ser and Asn
  VARIANT 22: Xaa22 is independently selected from Glu, Gln, Ser, Thr and Asn
  VARIANT 26: Xaa26 is independently selected from Pro, Arg and Ile
  VARIANT 31: Xaa31 is independently selected from Ser, Glu, Asp and Asn
  VARIANT 35: Xaa35 is independently selected from His, Arg, Lys, Asp and Glu
  VARIANT 37: Xaa37 is independently selected from Pro and Tyr

SEQ ID NO: 11 - protein, 37 aa, Artificial Sequence; identical to SEQ ID NO: 3
  Formula A1-4
  VARIANT 1: Xaa1 is independently selected from Ala, Cys, Glu, Gly, His, Arg, Ser and Lys
  VARIANT 3: Xaa3 is Asn
  VARIANT 14: Xaa14 is independently selected from Asp, Glu, His, Asn, Arg, Gly, Ala, Ser, Lys, Thr and Cys
  VARIANT 17: Xaa17 is independently selected from Arg and Val
  VARIANT 18: Xaa18 is His
  VARIANT 21: Xaa21 is Pro
  VARIANT 22: Xaa22 is Asn
  VARIANT 25: Xaa25 is independently selected from Pro and Ala
  VARIANT 26: Xaa26 is independently selected from Pro and Ile
  VARIANT 27: Xaa27 is independently selected from Pro and Leu
  VARIANT 28: Xaa28 is independently selected from Pro and Ser
  VARIANT 29: Xaa29 is independently selected from Pro and Ser
  VARIANT 31: Xaa31 is independently selected from Pro and Asn
  VARIANT 34: Xaa34 is independently selected from Pro, His, Lys, Arg and Ser
  VARIANT 35: Xaa35 is independently selected from Asp, Arg, Glu, Lys, His and Asn
  VARIANT 37: Xaa37 is independently selected from Pro and Tyr

SEQ ID NO: 12 - protein, 37 aa, Artificial Sequence
  Amylin RA Cpd 5
KCNTATCATQRLAEFLRHSSNNFGPILPPTNVGSNTP

SEQ ID NO: 13 - protein, 35 aa, Artificial Sequence
  Formula B1-1
  VARIANT 1: Xaa(-1) is absent or Glu
  VARIANT 2: Xaa1 is absent or selected from the group consisting of Glu or Ala
  VARIANT 3: Xaa2 is selected from the group consisting of Leu, Ala or Pro
  VARIANT 4: Xaa3 is selected from the group consisting of Ser or Pro
  VARIANT 5: Xaa4 is selected from the group consisting of Glu, Pro, Lys, Gln or Gly
  VARIANT 6: Xaa5 is selected from the group consisting of Leu, Val, or Ile
  VARIANT 7: Xaa6 is Ser, Thr or His
  VARIANT 8: Xaa7 is Thr
  VARIANT 9: Xaa8 is selected from the group consisting of Leu or Ala
  VARIANT 10: Xaa9 is selected from the group consisting of Ala, Val, Ile, Ser or Thr
  VARIANT 11: Xaa10 is selected from the group consisting of Leu, Ala, Ile, His or Val
  VARIANT 12: Xaa11 is Gly
  VARIANT 13: Xaa12 is selected from the group consisting of Arg, His or Lys
  VARIANT 14: Xaa13 is Leu
  VARIANT 15: Xaa14 is selected from the group consisting of Ser, Thr or Glu
  VARIANT 16: Xaa15 is selected from the group consisting of Ala, Gln, Glu, D-Glu or Thr
  VARIANT 17: Xaa16 is selected from the group consisting of Arg, Glu, Lys or Gln
  VARIANT 18: Xaa17 is selected from the group consisting of Leu or Ile
  VARIANT 19: Xaa18 is selected from the group consisting of His or Ala
  VARIANT 20: Xaa19 is selected from the group consisting of Glu, Arg or Lys
  VARIANT 21: Xaa20 is selected from the group consisting of Leu, Ile or Val
  VARIANT 22: Xaa21 is selected from the group consisting of Ala, Gln, Ser, Glu or Thr
  VARIANT 23: Xaa22 is Thr
  VARIANT 24: Xaa23 is selected from the group consisting of Thr, Tyr or Leu
  VARIANT 25: Xaa24 is Pro
  VARIANT 26: Xaa25 is selected from the group consisting of Arg, Pro, His or Lys
  VARIANT 27: Xaa26 is Thr
  VARIANT 28: Xaa27 is selected from the group consisting of Glu, Gln, Gly or Lys
  VARIANT 29: Xaa28 is selected from the group consisting of Thr or Pro
  VARIANT 30: Xaa29 is Gly
  VARIANT 31: Xaa30 is selected from the group consisting of Pro, Ser or Thr
  VARIANT 32: Xaa31 is selected from the group consisting of Glu, Gln, Gly, Ala, Pro or Lys
  VARIANT 33: Xaa32 is selected from the group consisting of Thr, Ser, His, Pro or Ala
  VARIANT 34: Xaa33 is selected from the group consisting of Pro, Tyr, His, Phe, Leu, Ser, Gly or Ala
  VARIANT 35: Xaa34 is absent or Gly
XXXXXXXXXXXXXXXXXXXXXXXXXXXXXXXXXXX

SEQ ID NO: 14 - protein, 36 aa, Artificial Sequence
  Formula B1-2
  VARIANT 1: Xaa1 is absent or selected from the group consisting of Glu or Ala
  VARIANT 2: Xaa2 is selected from the group consisting of Leu, Ala or Pro
  VARIANT 3: Xaa3 is selected from the group consisting of Ser or Pro
  VARIANT 4: Xaa4 is selected from the group consisting of Glu, Pro, Lys, Gln or Gly
  VARIANT 5: Xaa5 is selected from the group consisting of Leu, Val, or Ile
  VARIANT 6: Xaa6 is Ser, Thr or His
  VARIANT 7: Xaa7 is Thr
  VARIANT 8: Xaa8 is selected from the group consisting of Leu or Ala,
  VARIANT 9: Xaa9 is selected from the group consisting of Ala, Val, Ile, Ser or Thr
  VARIANT 10: Xaa10 is selected from the group consisting of Leu, Ala, Ile, His or Val
  VARIANT 11: Xaa11 is Gly
  VARIANT 12: Xaa12 is selected from the group consisting of Arg, His or Lys
  VARIANT 13: Xaa13 is Leu
  VARIANT 14: Xaa14 is selected from the group consisting of Ser, Thr or Glu
  VARIANT 15: Xaa15 is selected from the group consisting of Ala, Gln, Glu, D-Glu or Thr
  VARIANT 16: Xaa16 is selected from the group consisting of Arg, Glu, Lys or Gln
  VARIANT 17: Xaa17 is selected from the group consisting of Leu or Ile,
  VARIANT 18: Xaa18 is selected from the group consisting of His or Ala
  VARIANT 19: Xaa19 is selected from the group consisting of Glu, Arg or Lys
  VARIANT 20: Xaa20 is selected from the group consisting of Leu, Ile or Val
  VARIANT 21: Xaa21 is selected from the group consisting of Ala, Gln, Ser, Glu or Thr
  VARIANT 22: Xaa22 is Thr
  VARIANT 23: Xaa23 is selected from the group consisting of Thr, Tyr or Leu
  VARIANT 24: Xaa24 is Pro
  VARIANT 25: Xaa25 is selected from the group consisting of Arg, Pro, His or Lys,
  VARIANT 26: Xaa26 is Thr
  VARIANT 27: Xaa27 is selected from the group consisting of Glu, Gln, Gly or Lys
  VARIANT 28: Xaa28 is selected from the group consisting of Thr or Pro
  VARIANT 29: Xaa29 is Gly
  VARIANT 30: Xaa30 is selected from the group consisting of Pro, Ser or Thr
  VARIANT 31: Xaa31 is selected from the group consisting of Glu, Gln, Gly, Ala, Pro or Lys
  VARIANT 32: Xaa32 is selected from the group consisting of Thr, Ser, His, Pro or Ala
  VARIANT 33: Xaa33 is selected from the group consisting of Pro, Tyr, His, Phe, Leu, Ser, Gly or Ala
  VARIANT 34: Xaa34 is absent or Gly
  VARIANT 35: Xaa35 is absent or Thr
  VARIANT 36: Xaa36 is absent or Tyr
XXXXXXXXXXXXXXXXXXXXXXXXXXXXXXXXXXXX

SEQ ID NO: 15 - protein, 33 aa, Artificial Sequence
  Formula B1-3
  VARIANT 1: Xaa1 is absent or selected from the group consisting of Glu or Ala
  VARIANT 2: Xaa2 is selected from the group consisting of Leu, Ala or Pro
  VARIANT 3: Xaa3 is selected from the group consisting of Ser or Pro
  VARIANT 4: Xaa4 is selected from the group consisting of Glu, Pro, Lys, Gln or Gly
  VARIANT 5: Xaa5 is selected from the group consisting of Leu, Val, or Ile,
  VARIANT 6: Xaa6 is selected from the group consisting of Ser, Thr or His,
  VARIANT 8: Xaa8 is selected from the group consisting of Leu or Ala,
  VARIANT 9: Xaa9 is selected from the group consisting of Ala, Val, Ile, Ser or Thr
  VARIANT 10: Xaa10 is selected from the group consisting of Leu, Ala, Ile, His or Val
  VARIANT 12: Xaa12 is selected from the group consisting of Arg, His or Lys
  VARIANT 14: Xaa14 is selected from the group consisting of Ser, Thr or Glu
  VARIANT 15: Xaa15 is selected from the group consisting of Ala, Gln, Glu, D-Glu or Thr
  VARIANT 16: Xaa16 is selected from the group consisting of Arg, Glu, Lys or Gln
  VARIANT 17: Xaa17 is selected from the group consisting of Leu or Ile,
  VARIANT 18: Xaa18 is selected from the group consisting of His or Ala
  VARIANT 19: Xaa19 is selected from the group consisting of Glu, Arg or Lys
  VARIANT 20: Xaa20 is selected from the group consisting of Leu, Ile or Val
  VARIANT 21: Xaa21 is selected from the group consisting of Ala, Gln, Ser, Glu or Thr
  VARIANT 23: Xaa23 is selected from the group consisting of Thr, Tyr or Leu
  VARIANT 25: Xaa25 is selected from the group consisting of Arg, Pro, His or Lys
  VARIANT 27: Xaa27 is selected from the group consisting of Glu, Gln, Gly or Lys
  VARIANT 28: Xaa28 is selected from the group consisting of Thr or Pro
  VARIANT 30: Xaa30 is selected from the group consisting of Pro, Ser or Thr
  VARIANT 31: Xaa31 is selected from the group consisting of Glu, Gln, Gly, Ala, Pro or Lys
  VARIANT 32: Xaa32 is selected from the group consisting of Thr, Ser, His, Pro or Ala
  VARIANT 33: Xaa33 is selected from the group consisting of Pro, Tyr, His, Phe, Leu, Ser, Gly or Ala
XXXXXXTXXXGXLXXXXXXXXTXPXTXXGXXXX

SEQ ID NO: 16 - protein, 33 aa, Artificial Sequence
  Amylin RA Cpd 6
EASELSTAALGRLSAELHELATLPRTETGPESP

SEQ ID NO: 17 - protein, 33 aa, Artificial Sequence; identical to SEQ ID NO: 16
  Amylin RA 2

SEQ ID NO: 18 - protein, 33 aa, Artificial Sequence; identical to SEQ ID NO: 16
  Amylin RA 3

SEQ ID NO: 19 - protein, 38 aa, Artificial Sequence; identical to SEQ ID NO: 5
  Formula C1-1
  VARIANT 1: Xaa0 is a basic amino acid or is absent
  VARIANT 2: Xaa1 is a basic amino acid or is selected from the group consisting of Ala and Trp
  DISULFID 3..8
  VARIANT 4: Xaa3 is selected from the group consisting of Asn, Gly, Ser, Pro, Asp and Glu;
  VARIANT 11: Xaa10 is selected from the group consisting of Gln, Gly, Ala, Ser, Leu, Thr, Pro, Asp and Glu
  VARIANT 13: Xaa12 is selected from the group consisting of Leu and DLeu
  VARIANT 15: Xaa14 is selected from the group consisting of Glu, DGlu, Asp and DAsp
  VARIANT 17: Xaa16 is selected from the group consisting of Leu and DLeu, or is absent
  VARIANT 18: Xaa17 is selected from the group consisting of His, DHis, Val, DVal, Arg, DArg, Lys, DLys, Orn, DOrn, Dap and Dab, or is absent
  VARIANT 19: Xaa18 is selected from the group consisting of His, DHis, Arg, DArg, Dap and Dab, or is absent
  VARIANT 20: Xaa19 is selected from the group consisting of Ser and DSer, or is absent;
  VARIANT 21: Xaa20 is selected from the group consisting of Ser and DSer, or is absent
  VARIANT 22: Xaa21 is selected from the group consisting of Asn, DAsn, Glu, DGlu, Asp, DAsp, Ser and DSer, or is absent
  VARIANT 23: Xaa22 is selected from the group consisting of Asn, DAsn, Glu, DGlu, Asp, DAsp, Ser and DSer, or is absent
  VARIANT 24: Xaa23 is selected from the group consisting of Phe and DPhe, or is absent;
  VARIANT 25: Xaa24 is selected from the group consisting of Gly(Me), Ala(Me), DAla(Me), Ile(Me), DIle(Me), Ala, DAla, Pro and DPro,or is absent
  VARIANT 26: Xaa25 is selected from the group consisting of Ala, DAla, Pro and DPro, or is absent
  VARIANT 27: Xaa26 is selected from the group consisting of Gly(Me), Ile(Me), DIle(Me), Ile and DIle, or is absent
  VARIANT 28: Xaa27 is selected from the group consisting of Leu and DLeu, or is absent
  VARIANT 29: Xaa28 is selected from the group consisting of Ser, DSer, Pro, DPro, Ser(Me) and DSer(Me), or is absent
  VARIANT 30: Xaa29 is selected from the group consisting of Ser, DSer, Pro, DPro, Ser(Me) and DSer(Me), or is absent
  VARIANT 31: Xaa30 is selected from the group consisting of Thr and DThr, or is absent
  VARIANT 32: Xaa31 is selected from the group consisting of Asn, DAsn, Glu, DGlu, Asp and DAsp, or is absent
  VARIANT 36: Xaa35 is selected from the group consisting of His, DHis, Asn, DAsn, Glu, DGlu, Asp and DAsp, or is absent
  VARIANT 38: Xaa37 is selected from the group consisting of Tyr, DTyr, Pro, DPro, Hyp, Phe, Ser, Gly, Ala, Val, Ile, Leu, Thr, Tyr(Me), Gly(Me), Ala(Me), Ile(Me), Aze, Pip, Apr, Php and Bep, or is absent

SEQ ID NO: 20 - protein, 37 aa, Artificial Sequence
  Formula C1-2
  VARIANT 1: Xaa1 is a basic amino acid or is selected from the group consisting of Ala and Trp
  DISULFID 2..7
  VARIANT 3: Xaa3 is selected from the group consisting of Asn, Gly, Ser, Pro, Asp and Glu
  VARIANT 10: Xaa10 is selected from the group consisting of Gln, Gly, Ala, Ser, Leu, Thr, Pro, Asp and Glu
  VARIANT 12: Xaa12 is selected from the group consisting of Leu and DLeu
  VARIANT 14: Xaa14 is selected from the group consisting of Glu, DGlu, Asp and DAsp
  VARIANT 16: Xaa16 is selected from the group consisting of Leu and DLeu, or is absent
  VARIANT 17: Xaa17 is selected from the group consisting of His, DHis, Val, DVal, Arg, DArg, Lys, DLys, Orn, DOrn, Dap and Dab, or is absent
  VARIANT 18: Xaa18 is selected from the group consisting of His, DHis, Arg, DArg, Dap and Dab, or is absent
  VARIANT 19: Xaa19 is selected from the group consisting of Ser and DSer, or is absent
  VARIANT 20: Xaa20 is selected from the group consisting of Ser and DSer, or is absent
  VARIANT 21: Xaa21 is selected from the group consisting of Asn, DAsn, Glu, DGlu, Asp, DAsp, Ser and DSer, or is absent
  VARIANT 22: Xaa22 is selected from the group consisting of Asn, DAsn, Glu, DGlu, Asp, DAsp, Ser and DSer, or is absent
  VARIANT 23: Xaa23 is selected from the group consisting of Phe and DPhe, or is absent
  VARIANT 24: Xaa24 is selected from the group consisting of Gly(Me), Ala(Me), DAla(Me), Ile(Me), DIle(Me), Ala, DAla, Pro and DPro,or is absent
  VARIANT 25: Xaa25 is selected from the group consisting of Ala, DAla, Pro and DPro, or is absent
  VARIANT 26: Xaa26 is selected from the group consisting of Gly(Me), Ile(Me), DIle(Me), Ile and DIle, or is absent
  VARIANT 27: Xaa27 is selected from the group consisting of Leu and DLeu, or is absent
  VARIANT 28: Xaa28 is selected from the group consisting of Ser, DSer, Pro, DPro, Ser(Me) and DSer(Me), or is absent
  VARIANT 29: Xaa29 is selected from the group consisting of Ser, DSer, Pro, DPro, Ser(Me) and DSer(Me), or is absent
  VARIANT 30: Xaa30 is selected from the group consisting of Thr and DThr, or is absent
  VARIANT 31: Xaa31 is selected from the group consisting of Asn, DAsn, Glu, DGlu, Asp and DAsp, or is absent;
  VARIANT 35: Xaa35 is selected from the group consisting of His, DHis, Asn, DAsn, Glu, DGlu, Asp and DAsp, or is absent
  VARIANT 37: Xaa37 is selected from the group consisting of Tyr, DTyr, Pro, DPro, Hyp, Phe, Ser, Gly, Ala, Val, Ile, Leu, Thr, Tyr(Me), Gly(Me), Ala(Me), Ile(Me), Aze, Pip, Apr, Php and Bep, or is absent
XCXTATCATXRXAXFXXXXXXXXXXXXXXXXVGSXTX

SEQ ID NO: 21 - protein, 37 aa, Artificial Sequence
  Formula C1-3
  VARIANT 1: Xaa1 is selected from the group consisting of Trp, Lys and Arg
  DISULFID 2..7
  VARIANT 3: Xaa3 is selected from the group consisting of Gly, Asn, Glu and Pro;
  VARIANT 10: Xaa10 is selected from the group consisting of Gln, Asp and Glu
  VARIANT 14: Xaa14 is selected from the group consisting of Asp and Glu
  VARIANT 16: Xaa16 is Leu or is absent
  VARIANT 17: Xaa17 is His or is absent
  VARIANT 18: Xaa18 is selected from the group consisting of His and Arg, or is absent
  VARIANT 19: Xaa19 is selected from the group consisting of Ser and D-Ser, or is absent
  VARIANT 20: Xaa20 is Ser or is absent
  VARIANT 21: Xaa21 is selected from the group consisting of Asn and Ser, or is absent
  VARIANT 22: Xaa22 is selected from the group consisting of Asn and Ser, or is absent
  VARIANT 23: Xaa23 is selected from the group consisting of Phe and D-Phe, or is absent;
  VARIANT 24: Xaa24 is Gly(Me) or is absent
  VARIANT 25: Xaa25 is Ala or is absent
  VARIANT 26: Xaa26 is Ile(Me) or is absent
  VARIANT 27: Xaa27 is Leu or is absent
  VARIANT 28: Xaa28 is selected from the group consisting of Ser, Ser(Me), D-Ser and D-Ser(Me), or is absent
  VARIANT 29: Xaa29 is selected from the group consisting of Ser and Ser(Me) or is absent
  VARIANT 30: Xaa30 is Thr or is absent
  VARIANT 31: Xaa31 is selected from the group consisting of Asp, Glu and Asn
  VARIANT 35: Xaa35 is selected from the group consisting of Asp, Glu and Asn
  VARIANT 37: Xaa37 is selected from the group consisting of Tyr, Tyr(Me), Pro, Hyp, Apr, Aze, Pip, Php and Bep
XCXTATCATXRLAXFXXXXXXXXXXXXXXXXVGSXTX

SEQ ID NO: 22 - protein, 37 aa, Artificial Sequence
  Formula C1-4
  VARIANT 1: Xaa1 is selected from the group consisting of Trp, Lys and Arg
  DISULFID 2..7
  VARIANT 3: Xaa3 is selected from the group consisting of Gly, Asn and Pro
  VARIANT 10: Xaa10 is selected from the group consisting of Gln, Asp and Glu;
  VARIANT 18: Xaa18 is selected from the group consisting of His and Arg;
  VARIANT 21: Xaa21 is selected from the group consisting of Asn and Ser, or is absent
  VARIANT 22: Xaa22 is selected from the group consisting of Asn and Ser, or is absent
  VARIANT 23: Xaa23 is selected from the group consisting of Phe and D-Phe;
  MOD_RES 24: METHYLATION MeGly
  MOD_RES 26: METHYLATION MeIle
  VARIANT 28: Xaa28 is selected from the group consisting of Ser and D-Ser
  VARIANT 31: Xaa31 is selected from the group consisting of Asp, Glu and Asn
  VARIANT 35: Xaa35 is selected from the group consisting of Asp, Glu and Asn
  VARIANT 37: Xaa37 is selected from the group consisting of Pro and Hyp
XCXTATCATXRLAEFLHXSSXXXGAILXSTXVGSXTX

SEQ ID NO: 23 - protein, 37 aa, Artificial Sequence
  Formula C1-5
  VARIANT 1: Xaa1 is a basic amino acid
  DISULFID 2..7
  VARIANT 14: Xaa14 is selected from the group consisting of Glu, DGlu, Asp and DAsp;
  VARIANT 16: Xaa16 is selected from the group consisting of Leu and DLeu, or is absent
  VARIANT 17: Xaa17 is selected from the group consisting of His, DHis, Val, DVal, Arg, DArg, Dap and Dab, or is absent
  VARIANT 18: Xaa18 is selected from the group consisting of His, DHis, Arg, DArg, Dap and Dab, or is absent
  VARIANT 19: Xaa19 is selected from the group consisting of Ser and DSer, or is absent
  VARIANT 20: Xaa20 is selected from the group consisting of Ser and DSer, or is absent;
  VARIANT 21: Xaa21 is selected from the group consisting of Asn, DAsn, Glu, DGlu, Asp, DAsp, Ser and DSer, or is absent
  VARIANT 22: Xaa22 is selected from the group consisting of Asn, DAsn, Glu, DGlu, Asp, DAsp, Ser and DSer, or is absent
  VARIANT 23: Xaa23 is selected from the group consisting of Phe and DPhe, or is absent
  VARIANT 24: Xaa24 is selected from the group consisting of Pro, DPro, Ala, DAla, Ala(Me), DAla(Me), Gly(Me), Ile(Me) and DIle(Me), or is absent
  VARIANT 25: Xaa25 is selected from the group consisting of Ala, DAla, Pro and DPro, or is absent;
  VARIANT 26: Xaa26 is selected from the group consisting of Gly(Me), Ile(Me), DIle(Me) and DIle, or is absent
  VARIANT 27: Xaa27 is selected from the group consisting of Leu and DLeu, or is absent
  VARIANT 28: Xaa28 is selected from the group consisting of Pro, DPro, Ser, DSer, Ser(Me) and DSer(Me), or is absent
  VARIANT 29: Xaa29 is selected from the group consisting of Pro, DPro, Ser, DSer, Ser(Me) and DSer(Me), or is absent
  VARIANT 30: Xaa30 is selected from the group consisting of Thr and DThr, or is absent
  VARIANT 31: Xaa31 is selected from the group consisting of Asn, DAsn, Glu, D-Glu, Asp and DAsp, or is absent
  VARIANT 35: Xaa35 is selected from the group consisting of His, DHis, Asn, DAsn, Glu, DGlu, Asp and DAsp, or is absent
  VARIANT 37: Xaa37 is selected from the group consisting of Tyr, DTyr, Pro and DPro, or is absent
XCNTATCATQRLAXFXXXXXXXXXXXXXXXXVGSXTX

SEQ ID NO: 24 - protein, 35 aa, Artificial Sequence
  Amylin RA Cpd 7
  DISULFID 2..7
  MOD_RES 22: METHYLATION MeGly
  MOD_RES 24: METHYLATION MeIle
RCNTATCATQRLAEFLHRSSFGAILSSTEVGSETP

SEQ ID NO: 25 - protein, 37 aa, Artificial Sequence
  Amylin RA Cpd 8
  DISULFID 2..7
  MOD_RES 24: METHYLATION MeGly
  MOD_RES 26: METHYLATION MeIle
RCNTATCATQRLAEFLHRSSNNFGAILSSTNVGSNTP

SEQ ID NO: 26 - protein, 37 aa, Artificial Sequence; identical to SEQ ID NO: 6
  Formula D1-1
  VARIANT 3: Xaa3 is selected from the group consisting of Asn, Gly, Pro and Gln
  VARIANT 10: Xaa10 is selected from the group consisting of Gln, Asp and Glu
  VARIANT 14: Xaa14 is selected from the group consisting of Asp, His, Asn and Aad
  VARIANT 17: Xaa17 is selected from the group consisting of His, Asn, Gln, Glu, Thr, Val, Lys and Aad
  VARIANT 19..20: Xaa19-Xaa20 is selected from the group consisting of Ser-Ser, Val-Val, Ser-Val and Val-Ser, or is absent
  SITE 21..22: Xaa21-Xaa22 are absent
  MOD_RES 24: METHYLATION MeGly
  MOD_RES 26: METHYLATION MeIle
  VARIANT 31: Xaa31 is selected from the group consisting of Asp, Glu and Asn
  VARIANT 35: Xaa35 is selected from the group consisting of Asp, Glu, Asn, Ser, Phe, Orn, Aad, Gly and Thr
  VARIANT 37: Xaa37 is selected from the group consisting of Pro, Apr and Hyp

SEQ ID NO: 27 - protein, 37 aa, Artificial Sequence
  Formula D1-2
  VARIANT 3: Xaa3 is selected from the group consisting of Asn, Gly and Gln
  VARIANT 10: Xaa10 is selected from the group consisting of Gln, Asp and Glu;
  VARIANT 14: Xaa14 is selected from the group consisting of Asp, His and Aad
  VARIANT 17: Xaa17 is selected from the group consisting of His, Asn, Gln, Glu, Lys and Aad
  VARIANT 19..20: Xaa19-Xaa20 is Ser-Ser or is absent
  SITE 21..22: Xaa21-Xaa22 are absent
  MOD_RES 24: METHYLATION MeGly
  MOD_RES 26: METHYLATION MeIle
  VARIANT 35: Xaa35 is selected from the group consisting of Asp, Glu, Asn, Ser, Orn, Aad, Gly and Thr
  VARIANT 37: Xaa37 is selected from the group consisting of Pro and Hyp
RCXTATCATXRLAXFLXRXXXXFGAILSSTEVGSXTX

SEQ ID NO: 28 - protein, 37 aa, Artificial Sequence; identical to SEQ ID NO: 27
  Formula D1-3
  VARIANT 3: Xaa3 is selected from the group consisting of Asn, Gly and Gln
  VARIANT 10: Xaa10 is selected from the group consisting of Gln, Asp and Glu
  VARIANT 14: Xaa14 is selected from the group consisting of Asp, His and Aad
  VARIANT 17: Xaa17 is selected from the group consisting of His and Gln
  VARIANT 19..20: Xaa19-Xaa20 is Ser-Ser or is absent
  SITE 21..22: Xaa21-Xaa22 are absent
  MOD_RES 24: METHYLATION MeGly
  MOD_RES 26: METHYLATION MeIle
  VARIANT 35: Xaa35 is selected from the group consisting of Asp, Glu, Asn, Aad and Gly
  VARIANT 37: Xaa37 is selected from the group consisting of Pro and Hyp

SEQ ID NO: 29 - protein, 35 aa, Artificial Sequence
  Amylin RA Cpd9
  DISULFID 2..7
  MOD_RES 22: METHYLATION MeGly
  MOD_RES 24: METHYLATION MeIle
  VARIANT 35: Xaa35 is Hyp
RCGTATCATERLAHFLQRSSFGAILSSTEVGSNTX

SEQ ID NO: 30 - protein, 37 aa, Artificial Sequence; identical to SEQ ID NO: 7
  Formula E1-1
  VARIANT 1: Xaa1 is selected from the group consisting of Arg, Lys and Glu
  STRAND 2..7: Xaa2 and Xaa7 are amino acid residues whose side chains together form a lactam bridge
  VARIANT 3: Xaa3 is selected from the group consisting of Gly, Gln and Pro
  VARIANT 4: Xaa4 is selected from the group consisting of Thr and Glu
  VARIANT 5: Xaa5 is selected from the group consisting of Ala and Leu
  VARIANT 6: Xaa6 is selected from the group consisting of Thr and Ser
  VARIANT 10: Xaa10 is selected from the group consisting of Glu and Gln
  VARIANT 14: Xaa14 is selected from the group consisting of Aad, His, Asp, Asn and Arg;
  VARIANT 17: Xaa17 is selected from the group consisting of Gln, His and Thr
  VARIANT 19..20: Xaa19-Xaa20 is selected from Ser-Ser, Thr-Thr, Ala-Thr, Ala-Ala, Gly-Thr, Gly-Gly and Ala-Asn or is absent
  SITE 21..22: Xaa21-Xaa22 are absent
  MOD_RES 24: METHYLATION MeGly
  MOD_RES 26: METHYLATION MeIle
  VARIANT 27: Xaa27 is selected from the group consisting of Leu and Pro
  VARIANT 32: Xaa32 is selected from the group consisting of Val and Thr
  VARIANT 35: Xaa35 is selected from the group consisting of Asn and Ser
  VARIANT 37: Xaa37 is selected from the group consisting of Hyp and Pro

SEQ ID NO: 31 - protein, 37 aa, Artificial Sequence
  Formula E1-2
  VARIANT 1: Xaa1 is selected from the group consisting of Arg and Lys
  STRAND 2..7: Xaa2 and Xaa7 are amino acid residues whose side chains together form a lactam bridge
  VARIANT 10: Xaa10 is selected from the group consisting of Glu and Gln
  VARIANT 14: Xaa14 is selected from the group consisting of Aad, Asp and His
  VARIANT 19..20: Xaa19-Xaa20 is selected from Ser-Ser and Thr-Thr or is absent
  SITE 21..22: Xaa21-Xaa22 are absent
  MOD_RES 24: METHYLATION MeGly
  MOD_RES 26: METHYLATION MeIle
  VARIANT 27: Xaa27 is selected from the group consisting of Leu and Pro
  VARIANT 37: Xaa37 is Hyp
XXGTATXATXRLAXFLQRXXXXFGAIXSSTEVGSNTX

SEQ ID NO: 32 - protein, 35 aa, Artificial Sequence
  Amylin RA Cpd 10
  STRAND 2..7: Xaa2 and Xaa7 are amino acid residues whose side chains together form a lactam bridge
  MOD_RES 22: METHYLATION MeGly
  MOD_RES 24: METHYLATION MeIle
  VARIANT 35: Xaa35 is Hyp
RDGTATKATQRLADFLQRSSFGAILSSTEVGSNTX

SEQ ID NO: 33 - protein, 35 aa, Artificial Sequence
  Amylin RA Cpd 11
  STRAND 2..7: Xaa2 and Xaa7 are amino acid residues whose side chains together form a lactam bridge
  VARIANT 14: Xaa14 is Aad
  MOD_RES 22: METHYLATION MeGly
  MOD_RES 24: METHYLATION MeIle
  VARIANT 35: Xaa35 is Hyp
RDGTATKATERLAXFLQRSSFGAILSSTEVGSNTX

SEQ ID NO: 34 - protein, 35 aa, Artificial Sequence
  Amylin RA Cpd 12
  STRAND 2..7: Xaa2 and Xaa7 are amino acid residues whose side chains together form a lactam bridge
  VARIANT 14: Xaa14 is Aad
  MOD_RES 22: METHYLATION MeGly
  MOD_RES 24: METHYLATION MeIle
  VARIANT 35: Xaa35 is Hyp
RDGTATKATERLAXFLQRTTFGAILSSTEVGSNTX

SEQ ID NO: 35 - protein, 35 aa, Artificial Sequence
  Amylin RA Cpd 13
  STRAND 2..7: Xaa2 and Xaa7 are amino acid residues whose side chains together form a lactam bridge
  MOD_RES 22: METHYLATION MeGly
  MOD_RES 24: METHYLATION MeIle
  VARIANT 35: Xaa35 is Hyp
RDGTATKATERLAHFLQRSSFGAILSSTEVGSNTX

SEQ ID NO: 36 - protein, 35 aa, Artificial Sequence
  Amylin RA Cpd 14
  STRAND 2..7: Xaa2 and Xaa7 are amino acid residues whose side chains together form a lactam bridge
  VARIANT 14: Xaa14 is Aad
  MOD_RES 22: METHYLATION MeGly
  MOD_RES 24: METHYLATION MeIle
  VARIANT 35: Xaa35 is Hyp
KDGTATKATQRLAXFLQRSSFGAILSSTEVGSNTX

SEQ ID NO: 37 - protein, 39 aa, Artificial Sequence
  Exenatide
HGEGTFTSDLSKQMEEEAVRLFIEWLKNGGPSSGAPPPS

SEQ ID NO: 38 - protein, 44 aa, Artificial Sequence
  Lixisenatide
HGEGTFTSDLSKQMEEEAVRLFIEWLKNGGPSSGAPPSKKKKKK

SEQ ID NO: 39 - protein, 29 aa, Homo sapiens
  Human Glucagon
HSQGTFTSDYSKYLDSRRAQDFVQWLMNT

SEQ ID NO: 40 - protein, 29 aa, Artificial Sequence
  Dasiglucagon
  VARIANT 16: Xaa16 is Aib
HSQGTFTSDYSKYLDXARAEEFVKWLEST

SEQ ID NO: 41 - protein, 39 aa, Artificial Sequence
  GIP Formula 2
  VARIANT 1: Xaa1 is selected from the group consisting of Tyr and D-Tyr
  VARIANT 2: Xaa2 is selected from the group consisting of Aib, Ala, and D-Ala
  VARIANT 6: Xaa6 is selected from the group consisting of Phe, alpha-methyl-Phe, Iva, Leu, alpha-methyl-Leu, and alpha-methyl-Phe(2F);
  VARIANT 13: Xaa13 is selected from the group consisting of alpha-methyl-Leu, Ala, Leu, and Aib
  VARIANT 16: Xaa16 is selected from the group consisting of Lys, Glu, and Orn
  VARIANT 17: Xaa17 is Ile
  VARIANT 18: Xaa18 is selected from the group consisting of His, Ala, and Arg
  VARIANT 20: Xaa20 is selected from the group consisting of Aib and Gln
  VARIANT 21: Xaa21 is selected from the group consisting of Asp and Glu
  VARIANT 22: Xaa22 is selected from the group consisting of Phe and alpha-methyl-Phe
  VARIANT 24: Xaa24 is selected from the group consisting of Glu, Asn, Gln, and D-Glu
  VARIANT 25: X25 is selected from the group consisting of Tyr, 4-Pal, Trp, and alpha-methyl-Tyr
  VARIANT 26: Xaa26 is Leu
  VARIANT 28: Xaa28 is selected from the group consisting of Glu and Ala
  VARIANT 29: Xaa29 is selected from the group consisting of Gly, Ala, Gln, and Thr
XXEGTXISDYSIXLDXXXQXXXVXXXLXXGPSSGAPPPS

SEQ ID NO: 42 - protein, 39 aa, Artificial Sequence
  GIP RA Cpd 15
  VARIANT 2: Xaa2 is D-Ala
  VARIANT 20: Xaa20 is Aib
YXEGTFISDYSILLDKIAQXDFVNWLLAQGPSSGAPPPS

SEQ ID NO: 43 - protein, 39 aa, Artificial Sequence
  GIP RA Cpd 16
  VARIANT 2: Xaa2 is Aib
  MOD_RES 13: Xaa13 is alpha-methyl-Leu
  VARIANT 20: Xaa20 is Aib
  VARIANT 25: Xaa25 is 4-Pal
YXEGTFISDYSIXLDKIHQXDFVEXLLEAGPSSGAPPPS

SEQ ID NO: 44 - protein, 39 aa, Artificial Sequence
  GIP RA Cpd 17
  VARIANT 2: Xaa2 is Aib
  VARIANT 13: Xaa13 is alpha-methyl-Leu
  VARIANT 16: Xaa16 is Orn
  VARIANT 20: Xaa20 is Aib
  VARIANT 25: Xaa25 is 4-Pal
YXEGTFISDYSIXLDXIHQXDFVEXLLEAGPSSGAPPPS

SEQ ID NO: 45 - protein, 39 aa, Artificial Sequence
  GIP RA Cpd 18
  VARIANT 2: Xaa2 is Aib
  VARIANT 13: Xaa13 is alpha-methyl-Leu
  VARIANT 20: Xaa20 is Aib
YXEGTFISDYSIXLDKIHQXDFVEYLLEGGPSSGAPPPS

SEQ ID NO: 46 - protein, 39 aa, Artificial Sequence
  GIP RA Cpd 19
  VARIANT 2: Xaa2 is Aib
  VARIANT 13: Xaa13 is alpha-methyl-Leu
  VARIANT 16: Xaa16 is Orn
  VARIANT 20: Xaa20 is Aib
YXEGTFISDYSIXLDXIHQXDFVEYLLEGGPSSGAPPPS

SEQ ID NO: 47 - protein, 39 aa, Artificial Sequence
  GIP RA Cpd 20
  VARIANT 2: Xaa2 is Aib
  VARIANT 13: Xaa13 is alpha-methyl-Leu
  VARIANT 16: Xaa16 is Orn
  VARIANT 20: Xaa20 is Aib
  VARIANT 24: Xaa24 is D-Glu
YXEGTFISDYSIXLDXIHQXEFVXYLLEGGPSSGAPPPS

SEQ ID NO: 48 - protein, 30 aa, Artificial Sequence
  GIP Formula 3
  VARIANT 2: Xaa2 is Aib, Ala, D-Ala, Gly, Ser, N-Me-Ser, Ac3c, Ac4c or Ac5c
  VARIANT 10: Xaa10 is Tyr, Leu or Ser
  VARIANT 11: Xaa11 is Ser or Leu
  VARIANT 12: Xaa12 is Lys or Ile
  VARIANT 15: Xaa15 is Asp or Glu
  VARIANT 16: Xaa16 is Ser, Glu or Lys
  VARIANT 17: Xaa17 is Ile, Lys, Gln or Arg
  VARIANT 18: Xaa18 is His, Arg or Ala
  VARIANT 19: Xaa19 is Gln, Lys, Ala or Glu
  VARIANT 20: Xaa20 is Gln, Lys, Ala, His or Arg
  VARIANT 21: Xaa21 is Ala, Leu, Asp or Glu
  VARIANT 23: Xaa23 is Val or Ile
  VARIANT 24: Xaa24 is Asn or Glu
  VARIANT 25: Xaa25 is Tyr or Trp
  VARIANT 27: Xaa27 is Leu, Glu, Ser, Lys or Val
  VARIANT 28: Xaa28 is Ala, Ser or Arg
  VARIANT 29: Xaa29 is Aib, Gly, Ala, Gln, Thr, Ser or Lys or is absent
  VARIANT 30: Xaa30 is Lys-Gly, Gly-Pro-Ser-Ser-Gly-Ala-Pro-Pro-Pro-Ser, Gly-Pr o-Ser-Ser-Gly-Ala-Pro-Pro- Ser, Pro-Ser-Ser-Gly-Ala-Pro-Pro-Pro-S er, Pro-Ser-Ser-Gly-Ala-Pro-Pro-Ser, Gly-Lys-Lys- Asn-Asp-Trp-Lys -His-Asn-lle-Thr-Gln or absent
YXEGTFISDXXXELXXXXXXXFXXXLXXXX

SEQ ID NO: 49 - protein, 30 aa, Artificial Sequence
  GIP Formula 4
  VARIANT 2: Xaa2 is Aib, Ala, D-Ala or Gly
  VARIANT 12: Xaa12 is Lys or Ile
  VARIANT 15: Xaa15 is Asp or Glu
  VARIANT 16: Xaa16 is Ser, Glu or Lys
  VARIANT 17: Xaa17 is Ile, Lys, Gln or Arg
  VARIANT 18: Xaa18 is His, Arg or Ala
  VARIANT 19: Xaa19 is Gln or Ala
  VARIANT 20: Xaa20 is Gln, Lys, Ala, His or Arg
  VARIANT 21: Xaa21 is Ala, Asp or Glu
  VARIANT 23: Xaa23 is Ile or Val
  VARIANT 24: Xaa24 is Asn or Glu
  VARIANT 25: Xaa25 is Tyr or Trp
  VARIANT 27: Xaa27 is Leu, Glu, Ser, Lys or Val
  VARIANT 28: Xaa28 is Ala, Ser or Arg
  VARIANT 29: Xaa29 is Aib, Gly, Ala, Gln, Thr, Ser or Lys or is absent
  VARIANT 30: Xaa30 is Lys-Gly, Gly-Pro-Ser-Ser-Gly-Ala-Pro-Pro-Pro-, Gly-Pro-S er-Ser-Gly-Ala-Pro-Pro-Ser, Pro-Ser-Ser-Gly-Ala-Pro-Pro-Pro-Ser, Pro-Ser-Ser-Gly-Ala-Pro-Pro-Ser, Gly-Lys-Lys-Asn- Asp-Trp-Lys-His -Asn-lle-Thr-Gln or absent
YXEGTFISDYSXELXXXXXXXFXXXLXXXX

SEQ ID NO: 50 - protein, 30 aa, Artificial Sequence
  GIP Formula 5
  VARIANT 2: Xaa2 is Aib
  VARIANT 15: Xaa15 is Asp or Glu
  VARIANT 16: Xaa16 is Lys
  VARIANT 17: Xaa17 is Ile
  VARIANT 18: Xaa18 is His or Ala
  VARIANT 19: Xaa19 is Gln or Ala
  VARIANT 20: Xaa20 is Gln, Lys or Arg
  VARIANT 21: Xaa21 is Ala, Asp or Glu
  VARIANT 24: Xaa24 is Asn or Glu
  VARIANT 25: Xaa25 is Tyr or Trp
  VARIANT 28: Xaa28 is Ala, Ser or Arg
  VARIANT 29: Xaa29 is Gln or is absent
  VARIANT 30: Xaa30 is Lys-Gly, Gly-Pro-Ser-Ser-Gly-Ala-Pro-Pro-Pro-Ser, Gly-Pr o-Ser-Ser-Gly-Ala-Pro-Pro- Ser, Pro-Ser-Ser-Gly-Ala-Pro-Pro-Pro-S er, Pro-Ser-Ser-Gly-Ala-Pro-Pro-Ser, Gly-Lys-Lys- Asn-Asp-Trp-Lys -His-Asn-lle-Thr-Gln or absent
YXEGTFISDYSIELXXXXXXXFVXXLLAXX

SEQ ID NO: 51 - protein, 40 aa, Artificial Sequence
  GIP Formula 6
  VARIANT 2: Xaa2 represents Aib or D-Ala
  VARIANT 6: Xaa6 represents Iva, Phe, or Val
  VARIANT 7: Xaa7 represents Ile, Lys, or Val
  VARIANT 8: Xaa8 represents Ser
  VARIANT 9: Xaa9 represents Asp, Leu, or Phe
  VARIANT 10: Xaa10 represents Tyr
  VARIANT 11: Xaa11 represents Aib or Ser
  VARIANT 12: Xaa12 represents Ile
  VARIANT 13: Xaa13 represents Aib, Ala, Gln, Leu, Tyr, or D-Iva
  VARIANT 14: Xaa14 represents Leu
  VARIANT 15: Xaa15 represents Asp, Glu, Lys, Ser, or Tyr
  VARIANT 16: Xaa16 represents Arg or Lys
  VARIANT 17: Xaa17 represents Aib, Gln, or Ile
  VARIANT 18: Xaa18 represents Ala or His
  VARIANT 19: Xaa19 represents Gln or Ser
  VARIANT 20: Xaa20 represents Aib, Ala, or Gln
  VARIANT 21: Xaa21 represents Asn, Asp, Glu, Leu, or Ser
  VARIANT 22: Xaa22 represents Phe or alpha-methyl-Phe
  VARIANT 23: Xaa23 represents Ile or Val
  VARIANT 24: Xaa24 represents Arg, Asn, Asp, Lys, or Lys(Ac)
  VARIANT 25: Xaa25 represents Trp
  VARIANT 26: Xaa26 represents Aib, Iva, or Leu
  VARIANT 27: Xaa27 represents Leu
  VARIANT 28: Xaa28 represents Ala, Arg, Lys, or Lys(Ac)
  VARIANT 29: Xaa29 represents Gln or Gly
  VARIANT 30: Xaa30 represents Arg, Gly, or a deletion
  VARIANT 31: Xaa31 represents Pro or a deletion
  VARIANT 32: Xaa32 represents Ser or a deletion
  VARIANT 33: Xaa33 represents Ser or a deletion
  VARIANT 34: Xaa34 represents Gly or a deletion
  VARIANT 35: Xaa35 represents Ala or a deletion
  VARIANT 36: Xaa36 represents Pro or a deletion
  VARIANT 37: Xaa37 represents Pro or a deletion
  VARIANT 38: Xaa38 represents Pro or a deletion
  VARIANT 39: Xaa39 represents Lys, Ser, or a deletion
  VARIANT 40: Xaa40 represents Arg, Lys, or a deletion
YXEGTXXXXXXXXXXXXXXXXXXXXXXXXXXXXXXXXXXX

SEQ ID NO: 52 - protein, 36 aa, Artificial Sequence
  Peptide PYY (1-36)
YPIKPEAPGEDASPEELNRYYASLRHYLNLVTRQRY

SEQ ID NO: 53 - protein, 34 aa, Artificial Sequence
  Peptide PYY (3-36)
IKPEAPGEDASPEELNRYYASLRHYLNLVTRQRY

SEQ ID NO: 54 - protein, 33 aa, Artificial Sequence
  Peptide PYY (4-36)
KPEAPGEDASPEELNRYYASLRHYLNLVTRQRY